European Patent Specification EP 3 515 933 B9, published August 16, 2023. Title: Recombinant Binding Proteins. Applicant: Molecular Partners AG. The sequence listing filed with the application follows.

SEQUENCE LISTING (33 sequences)

SEQ ID NO: 1 - protein, 10 aa, Artificial Sequence
  His-tag
MRGSHHHHHH

SEQ ID NO: 2 - protein, 5 aa, Artificial Sequence
  GlySer linker
GGGGS

SEQ ID NO: 3 - protein, 7 aa, Artificial Sequence
  GlySer linker
GGGGSGS

SEQ ID NO: 4 - protein, 10 aa, Artificial Sequence
  GlySer linker
GGGGSGGGGS

SEQ ID NO: 5 - protein, 15 aa, Artificial Sequence
  GlySer linker
GGGGSGGGGSGGGGS

SEQ ID NO: 6 - protein, 20 aa, Artificial Sequence
  GlySer linker
GGGGSGGGGSGGGGSGGGGS

SEQ ID NO: 7 - protein, 8 aa, Artificial Sequence
  ProThr linker
GSPTPTPT

SEQ ID NO: 8 - protein, 15 aa, Artificial Sequence
  ProThr linker
GSPTPTPTTPTPTPT

SEQ ID NO: 9 - protein, 22 aa, Artificial Sequence
  ProThr linker
GSPTPTPTTPTPTPTTPTPTPT

SEQ ID NO: 10 - protein, 159 aa, Artificial Sequence
  Designed ankyrin repeat domain
GSDLGKKLLEAARAGQDDEVRILMANGADVNATDNDGYTPLHLAASNGHLEIVEVLLKNGADVNASDLTGITPLHLAAATGHLEIVEVLLKHGADVNAYDNDGHTPLHLAAKYGHLEIVEVLLKHGADVNAQDKFGKTAFDISIDNGNEDLAEILQKAA

SEQ ID NO: 11 - protein, 126 aa, Artificial Sequence
  Designed ankyrin repeat domain
GSDLGKKLLEAARAGQDDEVRILMANGADVNAKDKDGYTPLHLAAREGHLEIVEVLLKAGADVNAKDKDGYTPLHLAAREGHLEIVEVLLKAGADVNAQDKFGKTAFDISIDNGNEDLAEILQKAA

SEQ ID NO: 12 - protein, 126 aa, Artificial Sequence
  Designed ankyrin repeat domain
GSDLGKKLLEAARAGQDDEVRILLKAGADVNAKDYFSHTPLHLAARNGHLKIVEVLLKAGADVNAKDFAGKTPLHLAANDGHLEIVEVLLKAGADVNAQDIFGKTPADIAADAGHEDIAEVLQKAA

SEQ ID NO: 13 - protein, 126 aa, Artificial Sequence
  Designed ankyrin repeat domain
GSDLGKKLLEAARAGQDDEVRELLKAGADVNAKDYFSHTPLHLAARNGHLKIVEVLLKAGADVNAKDFAGKTPLHLAANDGHLEIVEVLLKAGADVNAQDIFGKTPADIAADAGHEDIAEVLQKAA

SEQ ID NO: 14 - protein, 126 aa, Artificial Sequence
  Designed ankyrin repeat domain
GSDLGKKLLEAARAGQDDEVRELLKAGADVNAKDYFSHTPLHLAARNGHLKIVEVLLKAGADVNAKDFAGKTPLHLAANEGHLEIVEVLLKAGADVNAQDIFGKTPADIAADAGHEDIAEVLQKAA

SEQ ID NO: 15 - protein, 126 aa, Artificial Sequence
  Designed ankyrin repeat domain
GSDLGKKLLEAARAGQDDEVRILMANGADVNAKDYFSHTPLHLAARNGHLKIVEVLLKAGADVNAKDFAGKTPLHLAANDGHLEIVEVLLKHGADVNAQDIFGKTPADIAADAGHEDIAEVLQKAA

SEQ ID NO: 16 - protein, 126 aa, Artificial Sequence
  Designed ankyrin repeat domain
GSDLGIKLLFAAAKGQDDEVRELLKAGADVNAKDFQGVTPLHIAAQSGHLEIVEVLLKAGADVNAKDVTGDTPLHLAAQHGHLEIVEVLLKAGADVNAQDERGWTPADLAADWGHEDIAEVLQKAA

SEQ ID NO: 17 - protein, 126 aa, Artificial Sequence
  Designed ankyrin repeat domain
GSDLGKKLLEAARAGQDDEVRELLKAGADVNAKDEYGLTPLYLATAHGHLEIVEVLLKAGADVNAVDAIGFTPLHLAAFIGHLEIAEVLLKAGADVNAQDKFGKTPADIAAGAGNEDIAEVLQKAA

SEQ ID NO: 18 - protein, 126 aa, Artificial Sequence
  Designed ankyrin repeat domain
GSDLGVKLLWAAARGQDDEVRELLKAGADVNAKDFQGITPLHIAATNGHLEIVEVLLKAGADVNAKDITGETPLHHAADSGHLEIVEVLLKAGADVNAQDKAGVTPADLAAAWGHEDIAEVLQKAA

SEQ ID NO: 19 - protein, 126 aa, Artificial Sequence
  Designed ankyrin repeat domain
GSDLGVKLLWAAARGQDDEVRILLAAGADVNAKDFQGITPLHIAAQSGHLEIVEVLLKAGADVNAKDVTGDTPLHLAAQHGHLVIVEVLLKAGADVNAQDERGWTPADLAADWGHEDIAEVLQKAA

SEQ ID NO: 20 - protein, 126 aa, Artificial Sequence
  Designed ankyrin repeat domain
GSDLGKKLLEAARAGQDDEVRILMANGADVNAKDEYGLTPLYLATAHGHLEIVEVLLKNGADVNAVDAIGFTPLHLAAFIGHLEIAEVLLKHGADVNAQDKFGKTAFDISIGNGNEDLAEILQKAA

SEQ ID NO: 21 - protein, 570 aa, Artificial Sequence
  Protein comprising four designed ankyrin repeat domains
GSDLGKKLLEAARAGQDDEVRELLKAGADVNAKDYFSHTPLHLAARNGHLKIVEVLLKAGADVNAKDFAGKTPLHLAANEGHLEIVEVLLKAGADVNAQDIFGKTPADIAADAGHEDIAEVLQKAAGSPTPTPTTPTPTPTTPTPTPTGSDLGIKLLFAAAKGQDDEVRELLKAGADVNAKDFQGVTPLHIAAQSGHLEIVEVLLKAGADVNAKDVTGDTPLHLAAQHGHLEIVEVLLKAGADVNAQDERGWTPADLAADWGHEDIAEVLQKAAGSPTPTPTTPTPTPTTPTPTPTGSDLGKKLLEAARAGQDDEVRELLKAGADVNAKDEYGLTPLYLATAHGHLEIVEVLLKAGADVNAVDAIGFTPLHLAAFIGHLEIAEVLLKAGADVNAQDKFGKTPADIAAGAGNEDIAEVLQKAAGSPTPTPTTPTPTPTTPTPTPTGSDLGKKLLEAARAGQDDEVRELLKAGADVNAKDYFSHTPLHLAARNGHLKIVEVLLKAGADVNAKDFAGKTPLHLAANEGHLEIVEVLLKAGADVNAQDIFGKTPADIAADAGHEDIAEVLQKAA

SEQ ID NO: 22 - protein, 570 aa, Artificial Sequence
  Protein comprising four designed ankyrin repeat domains
GSDLGKKLLEAARAGQDDEVRELLKAGADVNAKDYFSHTPLHLAARNGHLKIVEVLLKAGADVNAKDFAGKTPLHLAANDGHLEIVEVLLKAGADVNAQDIFGKTPADIAADAGHEDIAEVLQKAAGSPTPTPTTPTPTPTTPTPTPTGSDLGIKLLFAAAKGQDDEVRELLKAGADVNAKDFQGVTPLHIAAQSGHLEIVEVLLKAGADVNAKDVTGDTPLHLAAQHGHLEIVEVLLKAGADVNAQDERGWTPADLAADWGHEDIAEVLQKAAGSPTPTPTTPTPTPTTPTPTPTGSDLGKKLLEAARAGQDDEVRELLKAGADVNAKDEYGLTPLYLATAHGHLEIVEVLLKAGADVNAVDAIGFTPLHLAAFIGHLEIAEVLLKAGADVNAQDKFGKTPADIAAGAGNEDIAEVLQKAAGSPTPTPTTPTPTPTTPTPTPTGSDLGKKLLEAARAGQDDEVRELLKAGADVNAKDYFSHTPLHLAARNGHLKIVEVLLKAGADVNAKDFAGKTPLHLAANDGHLEIVEVLLKAGADVNAQDIFGKTPADIAADAGHEDIAEVLQKAA

SEQ ID NO: 23 - protein, 570 aa, Artificial Sequence
  Protein comprising four designed ankyrin repeat domains
GSDLGKKLLEAARAGQDDEVRELLKAGADVNAKDYFSHTPLHLAARNGHLKIVEVLLKAGADVNAKDFAGKTPLHLAANEGHLEIVEVLLKAGADVNAQDIFGKTPADIAADAGHEDIAEVLQKAAGSPTPTPTTPTPTPTTPTPTPTGSDLGVKLLWAAARGQDDEVRELLKAGADVNAKDFQGITPLHIAATNGHLEIVEVLLKAGADVNAKDITGETPLHHAADSGHLEIVEVLLKAGADVNAQDKAGVTPADLAAAWGHEDIAEVLQKAAGSPTPTPTTPTPTPTTPTPTPTGSDLGKKLLEAARAGQDDEVRELLKAGADVNAKDEYGLTPLYLATAHGHLEIVEVLLKAGADVNAVDAIGFTPLHLAAFIGHLEIAEVLLKAGADVNAQDKFGKTPADIAAGAGNEDIAEVLQKAAGSPTPTPTTPTPTPTTPTPTPTGSDLGKKLLEAARAGQDDEVRELLKAGADVNAKDYFSHTPLHLAARNGHLKIVEVLLKAGADVNAKDFAGKTPLHLAANEGHLEIVEVLLKAGADVNAQDIFGKTPADIAADAGHEDIAEVLQKAA

SEQ ID NO: 24 - protein, 570 aa, Artificial Sequence
  Protein comprising four designed ankyrin repeat domains
GSDLGKKLLEAARAGQDDEVRELLKAGADVNAKDYFSHTPLHLAARNGHLKIVEVLLKAGADVNAKDFAGKTPLHLAANEGHLEIVEVLLKAGADVNAQDIFGKTPADIAADAGHEDIAEVLQKAAGSPTPTPTTPTPTPTTPTPTPTGSDLGKKLLEAARAGQDDEVRELLKAGADVNAKDYFSHTPLHLAARNGHLKIVEVLLKAGADVNAKDFAGKTPLHLAANEGHLEIVEVLLKAGADVNAQDIFGKTPADIAADAGHEDIAEVLQKAAGSPTPTPTTPTPTPTTPTPTPTGSDLGIKLLFAAAKGQDDEVRELLKAGADVNAKDFQGVTPLHIAAQSGHLEIVEVLLKAGADVNAKDVTGDTPLHLAAQHGHLEIVEVLLKAGADVNAQDERGWTPADLAADWGHEDIAEVLQKAAGSPTPTPTTPTPTPTTPTPTPTGSDLGKKLLEAARAGQDDEVRELLKAGADVNAKDEYGLTPLYLATAHGHLEIVEVLLKAGADVNAVDAIGFTPLHLAAFIGHLEIAEVLLKAGADVNAQDKFGKTPADIAAGAGNEDIAEVLQKAA

SEQ ID NO: 25 - protein, 570 aa, Artificial Sequence
  Protein comprising four designed ankyrin repeat domains
GSDLGKKLLEAARAGQDDEVRELLKAGADVNAKDYFSHTPLHLAARNGHLKIVEVLLKAGADVNAKDFAGKTPLHLAANEGHLEIVEVLLKAGADVNAQDIFGKTPADIAADAGHEDIAEVLQKAAGSPTPTPTTPTPTPTTPTPTPTGSDLGKKLLEAARAGQDDEVRELLKAGADVNAKDYFSHTPLHLAARNGHLKIVEVLLKAGADVNAKDFAGKTPLHLAANEGHLEIVEVLLKAGADVNAQDIFGKTPADIAADAGHEDIAEVLQKAAGSPTPTPTTPTPTPTTPTPTPTGSDLGVKLLWAAARGQDDEVRELLKAGADVNAKDFQGITPLHIAATNGHLEIVEVLLKAGADVNAKDITGETPLHHAADSGHLEIVEVLLKAGADVNAQDKAGVTPADLAAAWGHEDIAEVLQKAAGSPTPTPTTPTPTPTTPTPTPTGSDLGKKLLEAARAGQDDEVRELLKAGADVNAKDEYGLTPLYLATAHGHLEIVEVLLKAGADVNAVDAIGFTPLHLAAFIGHLEIAEVLLKAGADVNAQDKFGKTPADIAAGAGNEDIAEVLQKAA

SEQ ID NO: 26 - protein, 562 aa, Artificial Sequence
  Protein comprising four designed ankyrin repeat domains
GSDLGKKLLEAARAGQDDEVRILMANGADVNAKDYFSHTPLHLAARNGHLKIVEVLLKAGADVNAKDFAGKTPLHLAANDGHLEIVEVLLKHGADVNAQDIFGKTPADIAADAGHEDIAEVLQKAAGGGGSGGGGSGGGGSGGGGSGSDLGAKLLSDLGVKLLWAAARGQDDEVRILLAAGADVNAKDFQGITPLHIAAQSGHLEIVEVLLKAGADVNAKDVTGDTPLHLAAQHGHLVIVEVLLKAGADVNAQDERGWTPADLAADWGHEDIAEVLQKAAGGGGSGGGGSGSDLGKKLLEAARAGQDDEVRILMANGADVNAKDEYGLTPLYLATAHGHLEIVEVLLKNGADVNAVDAIGFTPLHLAAFIGHLEIAEVLLKHGADVNAQDKFGKTAFDISIGNGNEDLAEILQKAAGGGGSGGGGSGGGGSGGGGSGSDLGKKLLEAARAGQDDEVRILMANGADVNAKDYFSHTPLHLAARNGHLKIVEVLLKAGADVNAKDFAGKTPLHLAANDGHLEIVEVLLKHGADVNAQDIFGKTPADIAADAGHEDIAEVLQKAA

SEQ ID NO: 27 - protein, 578 aa, Artificial Sequence
  Protein comprising four designed ankyrin repeat domains
GSDLGKKLLEAARAGQDDEVRILMANGADVNAKDYFSHTPLHLAARNGHLKIVEVLLKAGADVNAKDFAGKTPLHLAANDGHLEIVEVLLKHGADVNAQDIFGKTPADIAADAGHEDIAEVLQKAAGSPTPTPTTPTPTPTTPTPTPTGSDLGAKLLSDLGVKLLWAAARGQDDEVRILLAAGADVNAKDFQGITPLHIAAQSGHLEIVEVLLKAGADVNAKDVTGDTPLHLAAQHGHLVIVEVLLKAGADVNAQDERGWTPADLAADWGHEDIAEVLQKAAGSPTPTPTTPTPTPTTPTPTPTGSDLGKKLLEAARAGQDDEVRILMANGADVNAKDEYGLTPLYLATAHGHLEIVEVLLKNGADVNAVDAIGFTPLHLAAFIGHLEIAEVLLKHGADVNAQDKFGKTAFDISIGNGNEDLAEILQKAAGSPTPTPTTPTPTPTTPTPTPTGSDLGKKLLEAARAGQDDEVRILMANGADVNAKDYFSHTPLHLAARNGHLKIVEVLLKAGADVNAKDFAGKTPLHLAANDGHLEIVEVLLKHGADVNAQDIFGKTPADIAADAGHEDIAEVLQKAA

SEQ ID NO: 28 - protein, 283 aa, Artificial Sequence
  Protein comprising two designed ankyrin repeat domains
GSDLGIKLLFAAAKGQDDEVRELLKAGADVNAKDFQGVTPLHIAAQSGHLEIVEVLLKAGADVNAKDVTGDTPLHLAAQHGHLEIVEVLLKAGADVNAQDERGWTPADLAADWGHEDIAEVLQKAAGSPTPTPTTPTPTPTTPTPTPTGSDLGKKLLEAARAGQDDEVRELLKAGADVNAKDEYGLTPLYLATAHGHLEIVEVLLKAGADVNAVDAIGFTPLHLAAFIGHLEIAEVLLKAGADVNAQDKFGKTPADIAAGAGNEDIAEVLQKAAGGGSGGGSC

SEQ ID NO: 29 - protein, 414 aa, Artificial Sequence
  Protein comprising three designed ankyrin repeat domains
GSDLGKKLLEAARAGQDDEVRILMANGADVNAKDYFSHTPLHLAARNGHLKIVEVLLKAGADVNAKDFAGKTPLHLAANDGHLEIVEVLLKHGADVNAQDIFGKTPADIAADAGHEDIAEVLQKLGGGGSGGGGSGGGGSGGGGSRSDLGAKLLSDLGVKLLWAAARGQDDEVRILLAAGADVNAKDFQGITPLHIAAQSGHLEIVEVLLKAGADVNAKDVTGDTPLHLAAQHGHLVIVEVLLKAGADVNAQDERGWTPADLAADWGHEDIAEVLQKLGGGGSGGGGSRSDLGKKLLEAARAGQDDEVRILMANGADVNAKDEYGLTPLYLATAHGHLEIVEVLLKNGADVNAVDAIGFTPLHLAAFIGHLEIAEVLLKHGADVNAQDKFGKTAFDISIGNGNEDLAEILQKLN

SEQ ID NO: 30 - protein, 562 aa, Artificial Sequence
  Protein comprising four designed ankyrin repeat domains
GSDLGKKLLEAARAGQDDEVRILMANGADVNAKDYFSHTPLHLAARNGHLKIVEVLLKAGADVNAKDFAGKTPLHLAANDGHLEIVEVLLKHGADVNAQDIFGKTPADIAADAGHEDIAEVLQKAAGGGGSGGGGSGGGGSGGGGSGSDLGKKLLEAARAGQDDEVRILMANGADVNAKDYFSHTPLHLAARNGHLKIVEVLLKAGADVNAKDFAGKTPLHLAANDGHLEIVEVLLKHGADVNAQDIFGKTPADIAADAGHEDIAEVLQKAAGGGGSGGGGSGGGGSGGGGSGSDLGAKLLSDLGVKLLWAAARGQDDEVRILLAAGADVNAKDFQGITPLHIAAQSGHLEIVEVLLKAGADVNAKDVTGDTPLHLAAQHGHLVIVEVLLKAGADVNAQDERGWTPADLAADWGHEDIAEVLQKAAGGGGSGGGGSGSDLGKKLLEAARAGQDDEVRILMANGADVNAKDEYGLTPLYLATAHGHLEIVEVLLKNGADVNAVDAIGFTPLHLAAFIGHLEIAEVLLKHGADVNAQDKFGKTAFDISIGNGNEDLAEILQKAA

SEQ ID NO: 31 - protein, 580 aa, Artificial Sequence
  Protein comprising four designed ankyrin repeat domains
MRGSHHHHHHGSDLGKKLLEAARAGQDDEVRELLKAGADVNAKDYFSHTPLHLAARNGHLKIVEVLLKAGADVNAKDFAGKTPLHLAANEGHLEIVEVLLKAGADVNAQDIFGKTPADIAADAGHEDIAEVLQKAAGSPTPTPTTPTPTPTTPTPTPTGSDLGIKLLFAAAKGQDDEVRELLKAGADVNAKDFQGVTPLHIAAQSGHLEIVEVLLKAGADVNAKDVTGDTPLHLAAQHGHLEIVEVLLKAGADVNAQDERGWTPADLAADWGHEDIAEVLQKAAGSPTPTPTTPTPTPTTPTPTPTGSDLGKKLLEAARAGQDDEVRELLKAGADVNAKDEYGLTPLYLATAHGHLEIVEVLLKAGADVNAVDAIGFTPLHLAAFIGHLEIAEVLLKAGADVNAQDKFGKTPADIAAGAGNEDIAEVLQKAAGSPTPTPTTPTPTPTTPTPTPTGSDLGKKLLEAARAGQDDEVRELLKAGADVNAKDYFSHTPLHLAARNGHLKIVEVLLKAGADVNAKDFAGKTPLHLAANEGHLEIVEVLLKAGADVNAQDIFGKTPADIAADAGHEDIAEVLQKAA

SEQ ID NO: 32 - protein, 274 aa, Artificial Sequence
  Protein comprising two designed ankyrin repeat domains
GSDLGIKLLFAAAKGQDDEVRELLKAGADVNAKDFQGVTPLHIAAQSGHLEIVEVLLKAGADVNAKDVTGDTPLHLAAQHGHLEIVEVLLKAGADVNAQDERGWTPADLAADWGHEDIAEVLQKAAGSPTPTPTTPTPTPTTPTPTPTGSDLGKKLLEAARAGQDDEVRELLKAGADVNAKDEYGLTPLYLATAHGHLEIVEVLLKAGADVNAVDAIGFTPLHLAAFIGHLEIAEVLLKAGADVNAQDKFGKTPADIAAGAGNEDIAEVLQKAA

SEQ ID NO: 33 - protein, 422 aa, Artificial Sequence
  Protein comprising three designed ankyrin repeat domains
GSDLGKKLLEAARAGQDDEVRELLKAGADVNAKDYFSHTPLHLAARNGHLKIVEVLLKAGADVNAKDFAGKTPLHLAANEGHLEIVEVLLKAGADVNAQDIFGKTPADIAADAGHEDIAEVLQKAAGSPTPTPTTPTPTPTTPTPTPTGSDLGIKLLFAAAKGQDDEVRELLKAGADVNAKDFQGVTPLHIAAQSGHLEIVEVLLKAGADVNAKDVTGDTPLHLAAQHGHLEIVEVLLKAGADVNAQDERGWTPADLAADWGHEDIAEVLQKAAGSPTPTPTTPTPTPTTPTPTPTGSDLGKKLLEAARAGQDDEVRELLKAGADVNAKDEYGLTPLYLATAHGHLEIVEVLLKAGADVNAVDAIGFTPLHLAAFIGHLEIAEVLLKAGADVNAQDKFGKTPADIAAGAGNEDIAEVLQKAA